European Patent Application EP 4 163 374 A1, published April 12, 2023. Title: Tracking and Manipulating Cellular RNA via Nuclear Delivery of CRISPR/CAS9. Applicant: The Regents of the University of California. The sequence listing filed with the application follows.

SEQUENCE LISTING (39 sequences)

SEQ ID NO: 1 - RNA, 20 nt, synthetic construct
  misc_feature 1..20: note = Guide sequence
  source 1..20: mol_type = other RNA
ggactccccagcagtgaggg

SEQ ID NO: 2 - RNA, 20 nt, synthetic construct
  misc_feature 1..20: note = Guide sequence
  source 1..20: mol_type = other RNA
ggactccccagcagtgtccc

SEQ ID NO: 3 - RNA, 20 nt, synthetic construct
  misc_feature 1..20: note = Guide sequence
  source 1..20: mol_type = other RNA
ggactccccagctcactccc

SEQ ID NO: 4 - RNA, 20 nt, synthetic construct
  misc_feature 1..20: note = Guide sequence
  source 1..20: mol_type = other RNA
ggactcccgtcgtcactccc

SEQ ID NO: 5 - DNA, 39 bp, synthetic construct
  misc_feature 1..39: note = GAPDH mRNA 3'UTR
  source 1..39: mol_type = other DNA
cacaagaggaagagagagaccctcactgctggggagtcc

SEQ ID NO: 6 - DNA, 39 bp, synthetic construct
  misc_feature 1..39: note = Beta-actin mRNA 3'UTR
  source 1..39: mol_type = other DNA
gaaggtgacagcagtcggttggagcgagcatcccccaaa

SEQ ID NO: 7 - DNA, 39 bp, synthetic construct
  misc_feature 1..39: note = Gamma2 bacteriophage
  source 1..39: mol_type = other DNA
gctcaattttgacagcggtcatggcattccacttatcac

SEQ ID NO: 8 - RNA, 27 nt, synthetic construct
  modified_base 15: mod_base = OTHER; note = thymine
  modified_base 25: mod_base = OTHER; note = thymine
  misc_feature 1..27: note = PAMmer, beta-actin 3'UTR
  source 1..27: mol_type = other RNA
  modified_base 1: mod_base = OTHER; note = mU
  modified_base 3: mod_base = OTHER; note = mG
  modified_base 5: mod_base = OTHER; note = mU
  modified_base 7: mod_base = OTHER; note = mC
  modified_base 9: mod_base = OTHER; note = mU
  modified_base 12: mod_base = OTHER; note = mG
  modified_base 14: mod_base = OTHER; note = mC
  modified_base 16: mod_base = OTHER; note = mG
  modified_base 18: mod_base = OTHER; note = mU
  modified_base 20: mod_base = OTHER; note = mU
  modified_base 22: mod_base = OTHER; note = mA
  modified_base 24: mod_base = OTHER; note = mC
  modified_base 26: mod_base = OTHER; note = mU
tcgctccatgggactgctgtcaccttc

SEQ ID NO: 9 - DNA, 114 bp, synthetic construct
  misc_feature 1..114: note = sgRNA, beta-actin 3'UTR
  source 1..114: mol_type = other DNA
gtttgggggatgctcgctccagtttaagagctatgctggaaacagcatagcaagtttaaataaggctagtccgttatcaacttgaaaaagtggcaccgagtcggtgcttttttt

SEQ ID NO: 10 - RNA, 27 nt, synthetic construct
  modified_base 13: mod_base = OTHER; note = thymine
  modified_base 15: mod_base = OTHER; note = thymine
  modified_base 17: mod_base = OTHER; note = thymine
  modified_base 21: mod_base = OTHER; note = thymine
  modified_base 23: mod_base = OTHER; note = thymine
  misc_feature 1..27: note = PAMmer, GAPDH 3'UTR
  source 1..27: mol_type = other RNA
  modified_base 1: mod_base = OTHER; note = mA
  modified_base 3: mod_base = OTHER; note = mU
  modified_base 5: mod_base = OTHER; note = mA
  modified_base 7: mod_base = OTHER; note = mG
  modified_base 9: mod_base = OTHER; note = mC
  modified_base 12: mod_base = OTHER; note = mC
  modified_base 14: mod_base = OTHER; note = mC
  modified_base 16: mod_base = OTHER; note = mC
  modified_base 18: mod_base = OTHER; note = mU
  modified_base 20: mod_base = OTHER; note = mC
  modified_base 22: mod_base = OTHER; note = mC
  modified_base 24: mod_base = OTHER; note = mU
  modified_base 26: mod_base = OTHER; note = mU
agtgagggcggctctcttcctcttgtg

SEQ ID NO: 11 - DNA, 113 bp, synthetic construct
  misc_feature 1..113: note = sgRNA, GAPDH 3'UTR
  source 1..113: mol_type = other DNA
ggactccccagcagtgaggggtttaagagctatgctggaaacagcatagcaagtttaaataaggctagtccgttatcaacttgaaaaagtggcaccgagtcggtgcttttttt

SEQ ID NO: 12 - RNA, 27 nt, synthetic construct
  misc_feature 1..27: note = PAMmer, gamma2 bacteriophage
  source 1..27: mol_type = other RNA
  modified_base 2: mod_base = OTHER; note = thymine
  modified_base 23: mod_base = OTHER; note = thymine
  modified_base 1: mod_base = OTHER; note = mA
  modified_base 3: mod_base = OTHER; note = mG
  modified_base 5: mod_base = OTHER; note = mC
  modified_base 7: mod_base = OTHER; note = mU
  modified_base 9: mod_base = OTHER; note = mU
  modified_base 12: mod_base = OTHER; note = mG
  modified_base 14: mod_base = OTHER; note = mU
  modified_base 16: mod_base = OTHER; note = mU
  modified_base 18: mod_base = OTHER; note = mA
  modified_base 20: mod_base = OTHER; note = mA
  modified_base 22: mod_base = OTHER; note = mU
  modified_base 24: mod_base = OTHER; note = mG
  modified_base 26: mod_base = OTHER; note = mG
atgccatgtgggctgtcaaaattgagc

SEQ ID NO: 13 - DNA, 113 bp, synthetic construct
  misc_feature 1..113: note = sgRNA, gamma2 bacteriophage
  source 1..113: mol_type = other DNA
gtgataagtggaatgccatggtttaagagctatgctggaaacagcatagcaagtttaaataaggctagtccgttatcaacttgaaaaagtggcaccgagtcggtgcttttttt

SEQ ID NO: 14 - DNA, 21 bp, synthetic construct
  misc_feature 1..21: note = GAPDH forward primer
  source 1..21: mol_type = other DNA
aaggtgaaggtcggagtcaac

SEQ ID NO: 15 - DNA, 22 bp, synthetic construct
  misc_feature 1..22: note = GAPDH reverse primer
  source 1..22: mol_type = other DNA
ggggtcattgatggcaacaata

SEQ ID NO: 16 - DNA, 20 bp, synthetic construct
  misc_feature 1..20: note = Renilla luciferase forward primer
  source 1..20: mol_type = other DNA
gtaacgctgcctccagctac

SEQ ID NO: 17 - DNA, 20 bp, synthetic construct
  misc_feature 1..20: note = Renilla luciferase reverse primer
  source 1..20: mol_type = other DNA
gtggcccacaaagatgattt

SEQ ID NO: 18-19 - skipped (2 entries)

SEQ ID NO: 20 - DNA, 27 bp, synthetic construct
  misc_feature 1..27: note = PAMmer, CAG repeat
  source 1..27: mol_type = other DNA
  modified_base 1: mod_base = OTHER; note = mT
  modified_base 3: mod_base = OTHER; note = mC
  modified_base 5: mod_base = OTHER; note = mG
  modified_base 7: mod_base = OTHER; note = mT
  modified_base 9: mod_base = OTHER; note = mT
  modified_base 12: mod_base = OTHER; note = mC
  modified_base 14: mod_base = OTHER; note = mG
  modified_base 16: mod_base = OTHER; note = mT
  modified_base 18: mod_base = OTHER; note = mC
  modified_base 20: mod_base = OTHER; note = mG
  modified_base 22: mod_base = OTHER; note = mT
  modified_base 24: mod_base = OTHER; note = mC
  modified_base 26: mod_base = OTHER; note = mG
tgctgctgtggctgctgctgctgctgc

SEQ ID NO: 21 - RNA, 114 nt, synthetic construct
  misc_feature 1..114: note = sgRNA, CAG repeat
  source 1..114: mol_type = other RNA
  modified_base 2: mod_base = OTHER; note = thymine
  modified_base 5: mod_base = OTHER; note = thymine
  modified_base 8: mod_base = OTHER; note = thymine
  modified_base 11: mod_base = OTHER; note = thymine
  modified_base 14: mod_base = OTHER; note = thymine
  modified_base 17: mod_base = OTHER; note = thymine
  modified_base 20: mod_base = OTHER; note = thymine
gtgctgctgctgctgctgctggtttaagagctatgctggaaacagcatagcaagtttaaataaggctagtccgttatcaacttgaaaaagtggcaccgagtcggtgcttttttt

SEQ ID NO: 22 - DNA, 429 bp, synthetic construct
  misc_feature 1..429: note = U6 promoter-2xBbsi-sgRNA scaffold
  source 1..429: mol_type = other DNA
tgtacaaaaaagcaggctttaaaggaaccaattcagtcgactggatccggtaccaaggtcgggcaggaagagggcctatttcccatgattccttcatatttgcatatacgatacaaggctgttagagagataattagaattaatttgactgtaaacacaaagatattagtacaaaatacgtgacgtagaaagtaataatttcttgggtagtttgcagttttaaaattatgttttaaaatggactatcatatgcttaccgtaacttgaaagtatttcgatttcttggctttatatatcttgtggaaaggacgaaacaccgggtcttcgagaagacctgtttaagagctatgctggaaacagcatagcaagtttaaataaggctagtccgttatcaacttgaaaaagtggcaccgagtcggtgcttttttt

SEQ ID NO: 23 - DNA, 30 bp, synthetic construct
  misc_feature 1..30: note = CAG 10 probe
  source 1..30: mol_type = other DNA
cagcagcagcagcagcagcagcagcagcag

SEQ ID NO: 24 - protein, 154 aa, synthetic construct
  REGION 1..154: note = Split Venus (N-terminal portion, residues 2-155)(I152L reduced background complementation mutant)
VSKGEELFTGVVPILVELDGDVNGHKFSVSGEGEGDATYGKLTLKLICTTGKLPVPWPTLVTTLGYGLQCFARYPDHMKQHDFFKSAMPEGYVQERTIFFKDDGNYKTRAEVKFEGDTLVNRIELKGIDFKEDGNILGHKLEYNYNSHNVYLTA

SEQ ID NO: 25 - protein, 172 aa, synthetic construct
  REGION 1..172: note = Split Venus (N-terminal portion, residues 2-173)
VSKGEELFTGVVPILVELDGDVNGHKFSVSGEGEGDATYGKLTLKLICTTGKLPVPWPTLVTTLGYGLQCFARYPDHMKQHDFFKSAMPEGYVQERTIFFKDDGNYKTRAEVKFEGDTLVNRIELKGIDFKEDGNILGHKLEYNYNSHNVYITADKQKNGIKANFKIRHNIE

SEQ ID NO: 26 - protein, 99 aa, synthetic construct
  REGION 1..99: note = Split Venus (C-terminal portion, Feature of aa16-99 as residues 155-238)
ACKIPNDLKQKVMNHDKQKNGIKANFKIRHNIEDGGVQLADHYQQNTPIGDGPVLLPDNHYLSYQSKLSKDPNEKRDHMVLLEFVTAAGITLGMDELYK

SEQ ID NO: 27 - protein, 183 aa, synthetic construct
  REGION 1..183: note = PIN domain (from human SMG6)
QMELEIRPLFLVPDTNGFIDHLASLARLLESRKYILVVPLIVINELDGLAKGQETDHRAGGYARVVQEKARKSIEFLEQRFESRDSCLRALTSRGNELESIAFRSEDITGQLGNNDDLILSCCLHYCKDKAKDFMPASKEEPIRLLREVVLLTDDRNLRVKALTRNVPVRDIPAFLTWAQVGS

SEQ ID NO: 28 - protein, 418 aa, synthetic construct
  REGION 1..418: note = Human RBFOX1
MLASQGVLLHPYGVPMIVPAAPYLPGLIQGNQEAAAAPDTMAQPYASAQFAPPQNGIPAEYTAPHPHPAPEYTGQTTVPEHTLNLYPPAQTHSEQSPADTSAQTVSGTATQTDDAAPTDGQPQTQPSENTENKSQPKRLHVSNIPFRFRDPDLRQMFGQFGKILDVEIIFNERGSKGFGFVTFENSADADRAREKLHGTVVEGRKIEVNNATARVMTNKKTVNPYTNGWKLNPVVGAVYSPEFYAGTVLLCQANQEGSSMYSAPSSLVYTSAMPGFPYPAATAAAAYRGAHLRGRGRTVYNTFRAAAPPPPIPAYGGVVYQEPVYGNKLLQGGYAAYRYAQPTPATAAAYSDSYGRVYAADPYHHALAPAPTYGVGAMNAFAPLTDAKTRSHADDVGLVLSSLQASIYRGGYNRFAPY

SEQ ID NO: 29 - protein, 380 aa, synthetic construct
  REGION 1..380: note = Human RBFOX2
MEKKKMVTQGNQEPTTTPDAMVQPFTTIPFPPPPQNGIPTEYGVPHTQDYAGQTGEHNLTLYGSTQAHGEQSSNSPSTQNGSLTTEGGAQTDGQQSQTQSSENSESKSTPKRLHVSNIPFRFRDPDLRQMFGQFGKILDVEIIFNERGSKGFGFVTFENSADADRAREKLHGTVVEGRKIEVNNATARVMTNKKMVTPYANGWKLSPVVGAVYGPELYAASSFQADVSLGNDAAVPLSGRGGINTYIPLISLPLVPGFPYPTAATTAAAFRGAHLRGRGRTVYGAVRAVPPTAIPAYPGVVYQDGFYGADLYGGYAAYRYAQPATATAATAAAAAAAAYSDGYGRVYTADPYHALAPAASYGVGAVASLYRGGYSRFAPY

SEQ ID NO: 30 - protein, 238 aa, synthetic construct
  REGION 1..238: note = EGFP
VSKGEELFTGVVPILVELDGDVNGHKFSVSGEGEGDATYGKLTLKFICTTGKLPVPWPTLVTTLTYGVQCFSRYPDHMKQHDFFKSAMPEGYVQERTIFFKDDGNYKTRAEVKFEGDTLVNRIELKGIDFKEDGNILGHKLEYNYNSHNVYIMADKQKNGIKVNFKIRHNIEDGSVQLADHYQQNTPIGDGPVLLPDNHYLSTQSALSKDPNEKRDHMVLLEFVTAAGITLGMDELYK

SEQ ID NO: 31 - protein, 1382 aa, Streptococcus pyogenes
RTMDKKYSIGLAIGTNSVGWAVITDEYKVPSKKFKVLGNTDRHSIKKNLIGALLFDSGETAEATRLKRTARRRYTRRKNRICYLQEIFSNEMAKVDDSFFHRLEESFLVEEDKKHERHPIFGNIVDEVAYHEKYPTIYHLRKKLVDSTDKADLRLIYLALAHMIKFRGHFLIEGDLNPDNSDVDKLFIQLVQTYNQLFEENPINASGVDAKAILSARLSKSRRLENLIAQLPGEKKNGLFGNLIALSLGLTPNFKSNFDLAEDAKLQLSKDTYDDDLDNLLAQIGDQYADLFLAAKNLSDAILLSDILRVNTEITKAPLSASMIKRYDEHHQDLTLLKALVRQQLPEKYKEIFFDQSKNGYAGYIDGGASQEEFYKFIKPILEKMDGTEELLVKLNREDLLRKQRTFDNGSIPHQIHLGELHAILRRQEDFYPFLKDNREKIEKILTFRIPYYVGPLARGNSRFAWMTRKSEETITPWNFEEVVDKGASAQSFIERMTNFDKNLPNEKVLPKHSLLYEYFTVYNELTKVKYVTEGMRKPAFLSGEQKKAIVDLLFKTNRKVTVKQLKEDYFKKIECFDSVEISGVEDRFNASLGTYHDLLKIIKDKDFLDNEENEDILEDIVLTLTLFEDREMIEERLKTYAHLFDDKVMKQLKRRRYTGWGRLSRKLINGIRDKQSGKTILDFLKSDGFANRNFMQLIHDDSLTFKEDIQKAQVSGQGDSLHEHIANLAGSPAIKKGILQTVKVVDELVKVMGRHKPENIVIEMARENQTTQKGQKNSRERMKRIEEGIKELGSQILKEHPVENTQLQNEKLYLYYLQNGRDMYVDQELDINRLSDYDVDAIVPQSFLKDDSIDNKVLTRSDKNRGKSDNVPSEEVVKKMKNYWRQLLNAKLITQRKFDNLTKAERGGLSELDKAGFIKRQLVETRQITKHVAQILDSRMNTKYDENDKLIREVKVITLKSKLVSDFRKDFQFYKVREINNYHHAHDAYLNAVVGTALIKKYPKLESEFVYGDYKVYDVRKMIAKSEQEIGKATAKYFFYSNIMNFFKTEITLANGEIRKRPLIETNGETGEIVWDKGRDFATVRKVLSMPQVNIVKKTEVQTGGFSKESILPKRNSDKLIARKKDWDPKKYGGFDSPTVAYSVLVVAKVEKGKSKKLKSVKELLGITIMERSSFEKNPIDFLEAKGYKEVKKDLIIKLPKYSLFELENGRKRMLASAGELQKGNELALPSKYVNFLYLASHYEKLKGSPEDNEQKQLFVEQHKHYLDEIIEQISEFSKRVILADANLDKVLSAYNKHRDKPIREQAENIIHLFTLTNLGAPAAFKYFDTTIDRKRYTSTKEVLDATLIHQSITGLYETRIDLSQLGGDAYPYDVPDYASL

SEQ ID NO: 32 - protein, 1641 aa, synthetic construct
  REGION 1..1641: note = dCas9-2xNLS-EGFP
RTMDKKYSIGLAIGTNSVGWAVITDEYKVPSKKFKVLGNTDRHSIKKNLIGALLFDSGETAEATRLKRTARRRYTRRKNRICYLQEIFSNEMAKVDDSFFHRLEESFLVEEDKKHERHPIFGNIVDEVAYHEKYPTIYHLRKKLVDSTDKADLRLIYLALAHMIKFRGHFLIEGDLNPDNSDVDKLFIQLVQTYNQLFEENPINASGVDAKAILSARLSKSRRLENLIAQLPGEKKNGLFGNLIALSLGLTPNFKSNFDLAEDAKLQLSKDTYDDDLDNLLAQIGDQYADLFLAAKNLSDAILLSDILRVNTEITKAPLSASMIKRYDEHHQDLTLLKALVRQQLPEKYKEIFFDQSKNGYAGYIDGGASQEEFYKFIKPILEKMDGTEELLVKLNREDLLRKQRTFDNGSIPHQIHLGELHAILRRQEDFYPFLKDNREKIEKILTFRIPYYVGPLARGNSRFAWMTRKSEETITPWNFEEVVDKGASAQSFIERMTNFDKNLPNEKVLPKHSLLYEYFTVYNELTKVKYVTEGMRKPAFLSGEQKKAIVDLLFKTNRKVTVKQLKEDYFKKIECFDSVEISGVEDRFNASLGTYHDLLKIIKDKDFLDNEENEDILEDIVLTLTLFEDREMIEERLKTYAHLFDDKVMKQLKRRRYTGWGRLSRKLINGIRDKQSGKTILDFLKSDGFANRNFMQLIHDDSLTFKEDIQKAQVSGQGDSLHEHIANLAGSPAIKKGILQTVKVVDELVKVMGRHKPENIVIEMARENQTTQKGQKNSRERMKRIEEGIKELGSQILKEHPVENTQLQNEKLYLYYLQNGRDMYVDQELDINRLSDYDVDAIVPQSFLKDDSIDNKVLTRSDKNRGKSDNVPSEEVVKKMKNYWRQLLNAKLITQRKFDNLTKAERGGLSELDKAGFIKRQLVETRQITKHVAQILDSRMNTKYDENDKLIREVKVITLKSKLVSDFRKDFQFYKVREINNYHHAHDAYLNAVVGTALIKKYPKLESEFVYGDYKVYDVRKMIAKSEQEIGKATAKYFFYSNIMNFFKTEITLANGEIRKRPLIETNGETGEIVWDKGRDFATVRKVLSMPQVNIVKKTEVQTGGFSKESILPKRNSDKLIARKKDWDPKKYGGFDSPTVAYSVLVVAKVEKGKSKKLKSVKELLGITIMERSSFEKNPIDFLEAKGYKEVKKDLIIKLPKYSLFELENGRKRMLASAGELQKGNELALPSKYVNFLYLASHYEKLKGSPEDNEQKQLFVEQHKHYLDEIIEQISEFSKRVILADANLDKVLSAYNKHRDKPIREQAENIIHLFTLTNLGAPAAFKYFDTTIDRKRYTSTKEVLDATLIHQSITGLYETRIDLSQLGGDAYPYDVPDYASLGSGSPKKKRKVEDPKKKRKVDVSKGEELFTGVVPILVELDGDVNGHKFSVSGEGEGDATYGKLTLKFICTTGKLPVPWPTLVTTLTYGVQCFSRYPDHMKQHDFFKSAMPEGYVQERTIFFKDDGNYKTRAEVKFEGDTLVNRIELKGIDFKEDGNILGHKLEYNYNSHNVYIMADKQKNGIKVNFKIRHNIEDGSVQLADHYQQNTPIGDGPVLLPDNHYLSTQSALSKDPNEKRDHMVLLEFVTAAGITLGMDELYK

SEQ ID NO: 33 - protein, 1599 aa, synthetic construct
  REGION 1..1599: note = PIN-XTEN-dCas9-2xNLS
QMELEIRPLFLVPDTNGFIDHLASLARLLESRKYILVVPLIVINELDGLAKGQETDHRAGGYARVVQEKARKSIEFLEQRFESRDSCLRALTSRGNELESIAFRSEDITGQLGNNDDLILSCCLHYCKDKAKDFMPASKEEPIRLLREVVLLTDDRNLRVKALTRNVPVRDIPAFLTWAQVGSGSETPGTSESATPESDKKYSIGLAIGTNSVGWAVITDEYKVPSKKFKVLGNTDRHSIKKNLIGALLFDSGETAEATRLKRTARRRYTRRKNRICYLQEIFSNEMAKVDDSFFHRLEESFLVEEDKKHERHPIFGNIVDEVAYHEKYPTIYHLRKKLVDSTDKADLRLIYLALAHMIKFRGHFLIEGDLNPDNSDVDKLFIQLVQTYNQLFEENPINASGVDAKAILSARLSKSRRLENLIAQLPGEKKNGLFGNLIALSLGLTPNFKSNFDLAEDAKLQLSKDTYDDDLDNLLAQIGDQYADLFLAAKNLSDAILLSDILRVNTEITKAPLSASMIKRYDEHHQDLTLLKALVRQQLPEKYKEIFFDQSKNGYAGYIDGGASQEEFYKFIKPILEKMDGTEELLVKLNREDLLRKQRTFDNGSIPHQIHLGELHAILRRQEDFYPFLKDNREKIEKILTFRIPYYVGPLARGNSRFAWMTRKSEETITPWNFEEVVDKGASAQSFIERMTNFDKNLPNEKVLPKHSLLYEYFTVYNELTKVKYVTEGMRKPAFLSGEQKKAIVDLLFKTNRKVTVKQLKEDYFKKIECFDSVEISGVEDRFNASLGTYHDLLKIIKDKDFLDNEENEDILEDIVLTLTLFEDREMIEERLKTYAHLFDDKVMKQLKRRRYTGWGRLSRKLINGIRDKQSGKTILDFLKSDGFANRNFMQLIHDDSLTFKEDIQKAQVSGQGDSLHEHIANLAGSPAIKKGILQTVKVVDELVKVMGRHKPENIVIEMARENQTTQKGQKNSRERMKRIEEGIKELGSQILKEHPVENTQLQNEKLYLYYLQNGRDMYVDQELDINRLSDYDVDAIVPQSFLKDDSIDNKVLTRSDKNRGKSDNVPSEEVVKKMKNYWRQLLNAKLITQRKFDNLTKAERGGLSELDKAGFIKRQLVETRQITKHVAQILDSRMNTKYDENDKLIREVKVITLKSKLVSDFRKDFQFYKVREINNYHHAHDAYLNAVVGTALIKKYPKLESEFVYGDYKVYDVRKMIAKSEQEIGKATAKYFFYSNIMNFFKTEITLANGEIRKRPLIETNGETGEIVWDKGRDFATVRKVLSMPQVNIVKKTEVQTGGFSKESILPKRNSDKLIARKKDWDPKKYGGFDSPTVAYSVLVVAKVEKGKSKKLKSVKELLGITIMERSSFEKNPIDFLEAKGYKEVKKDLIIKLPKYSLFELENGRKRMLASAGELQKGNELALPSKYVNFLYLASHYEKLKGSPEDNEQKQLFVEQHKHYLDEIIEQISEFSKRVILADANLDKVLSAYNKHRDKPIREQAENIIHLFTLTNLGAPAAFKYFDTTIDRKRYTSTKEVLDATLIHQSITGLYETRIDLSQLGGDAYPYDVPDYASLGSGSPKKKRKVEDPKKKRKVDV

SEQ ID NO: 34 - protein, 1419 aa, synthetic construct
  REGION 1..1419: note = Telomerase-binding protein EST1A encoded by SMG6gene
MAEGLERVRISASELRGILATLAPQAGSRENMKELKEARPRKDNRRPDLEIYKPGLSRLRNKPKIKEPPGSEEFKDEIVNDRDCSAVENGTQPVKDVCKELNNQEQNGPIDPENNRGQESFPRTAGQEDRSLKIIKRTKKPDLQIYQPGRRLQTVSKESASRVEEEEVLNQVEQLRVEEDECRGNVAKEEVANKPDRAEIEKSPGGGRVGAAKGEKGKRMGKGEGVRETHDDPARGRPGSAKRYSRSDKRRNRYRTRSTSSAGSNNSAEGAGLTDNGCRRRRQDRTKERPRLKKQVSVSSTDSLDEDRIDEPDGLGPRRSSERKRHLERNWSGRGEGEQKNSAKEYRGTLRVTFDAEAMNKESPMVRSARDDMDRGKPDKGLSSGGKGSEKQESKNPKQELRGRGRGILILPAHTTLSVNSAGSPESAPLGPRLLFGSGSKGSRSWGRGGTTRRLWDPNNPDQKPALKTQTPQLHFLDTDDEVSPTSWGDSRQAQASYYKFQNSDNPYYYPRTPGPASQYPYTGYNPLQYPVGPTNGVYPGPYYPGYPTPSGQYVCSPLPTSTMSPEEVEQHMRNLQQQELHRLLRVADNQELQLSNLLSRDRISPEGLEKMAQLRAELLQLYERCILLDIEFSDNQNVDQILWKNAFYQVIEKFRQLVKDPNVENPEQIRNRLLELLDEGSDFFDSLLQKLQVTYKFKLEDYMDGLAIRSKPLRKTVKYALISAQRCMICQGDIARYREQASDTANYGKARSWYLKAQHIAPKNGRPYNQLALLAVYTRRKLDAVYYYMRSLAASNPILTAKESLMSLFEETKRKAEQMEKKQHEEFDLSPDQWRKGKKSTFRHVGDDTTRLEIWIHPSHPRSSQGTESGKDSEQENGLGSLSPSDLNKRFILSFLHAHGKLFTRIGMETFPAVAEKVLKEFQVLLQHSPSPIGSTRMLQLMTINMFAVHNSQLKDCFSEECRSVIQEQAAALGLAMFSLLVRRCTCLLKESAKAQLSSPEDQDDQDDIKVSSFVPDLKELLPSVKVWSDWMLGYPDTWNPPPTSLDLPSHVAVDVWSTLADFCNILTAVNQSEVPLYKDPDDDLTLLILEEDRLLSGFVPLLAAPQDPCYVEKTSDKVIAADCKRVTVLKYFLEALCGQEEPLLAFKGGKYVSVAPVPDTMGKEMGSQEGTRLEDEEEDVVIEDFEEDSEAEGSGGEDDIRELRAKKLALARKIAEQQRRQEKIQAVLEDHSQMRQMELEIRPLFLVPDTNGFIDHLASLARLLESRKYILVVPLIVINELDGLAKGQETDHRAGGYARVVQEKARKSIEFLEQRFESRDSCLRALTSRGNELESIAFRSEDITGQLGNNDDLILSCCLHYCKDKAKDFMPASKEEPIRLLREVVLLTDDRNLRVKALTRNVPVRDIPAFLTWAQVG

SEQ ID NO: 35 - protein, 152 aa, synthetic construct
  REGION 1..152: note = PIN domain
LFLVPDTNGFIDHLASLARLLESRKYILVVPLIVINELDGLAKGQETDHRAGGYARVVQEKARKSIEFLEQRFESRDSCLRALTSRGNELESIAFRSEDITGQLGNNDDLILSCCLHYCKDKAKDFMPASKEEPIRLLREVVLLTDDRNLRV

SEQ ID NO: 36 - protein, 16 aa, synthetic construct
  REGION 1..16: note = XTEN linker
SGSETPGTSESATPES

SEQ ID NO: 37 - protein, 1600 aa, synthetic construct
  REGION 1..1600: note = PIN-XTEN-dCas9
MQMELEIRPLFLVPDTNGFIDHLASLARLLESRKYILVVPLIVINELDGLAKGQETDHRAGGYARVVQEKARKSIEFLEQRFESRDSCLRALTSRGNELESIAFRSEDITGQLGNNDDLILSCCLHYCKDKAKDFMPASKEEPIRLLREVVLLTDDRNLRVKALTRNVPVRDIPAFLTWAQVGSGSETPGTSESATPESDKKYSIGLAIGTNSVGWAVITDEYKVPSKKFKVLGNTDRHSIKKNLIGALLFDSGETAEATRLKRTARRRYTRRKNRICYLQEIFSNEMAKVDDSFFHRLEESFLVEEDKKHERHPIFGNIVDEVAYHEKYPTIYHLRKKLVDSTDKADLRLIYLALAHMIKFRGHFLIEGDLNPDNSDVDKLFIQLVQTYNQLFEENPINASGVDAKAILSARLSKSRRLENLIAQLPGEKKNGLFGNLIALSLGLTPNFKSNFDLAEDAKLQLSKDTYDDDLDNLLAQIGDQYADLFLAAKNLSDAILLSDILRVNTEITKAPLSASMIKRYDEHHQDLTLLKALVRQQLPEKYKEIFFDQSKNGYAGYIDGGASQEEFYKFIKPILEKMDGTEELLVKLNREDLLRKQRTFDNGSIPHQIHLGELHAILRRQEDFYPFLKDNREKIEKILTFRIPYYVGPLARGNSRFAWMTRKSEETITPWNFEEVVDKGASAQSFIERMTNFDKNLPNEKVLPKHSLLYEYFTVYNELTKVKYVTEGMRKPAFLSGEQKKAIVDLLFKTNRKVTVKQLKEDYFKKIECFDSVEISGVEDRFNASLGTYHDLLKIIKDKDFLDNEENEDILEDIVLTLTLFEDREMIEERLKTYAHLFDDKVMKQLKRRRYTGWGRLSRKLINGIRDKQSGKTILDFLKSDGFANRNFMQLIHDDSLTFKEDIQKAQVSGQGDSLHEHIANLAGSPAIKKGILQTVKVVDELVKVMGRHKPENIVIEMARENQTTQKGQKNSRERMKRIEEGIKELGSQILKEHPVENTQLQNEKLYLYYLQNGRDMYVDQELDINRLSDYDVDAIVPQSFLKDDSIDNKVLTRSDKNRGKSDNVPSEEVVKKMKNYWRQLLNAKLITQRKFDNLTKAERGGLSELDKAGFIKRQLVETRQITKHVAQILDSRMNTKYDENDKLIREVKVITLKSKLVSDFRKDFQFYKVREINNYHHAHDAYLNAVVGTALIKKYPKLESEFVYGDYKVYDVRKMIAKSEQEIGKATAKYFFYSNIMNFFKTEITLANGEIRKRPLIETNGETGEIVWDKGRDFATVRKVLSMPQVNIVKKTEVQTGGFSKESILPKRNSDKLIARKKDWDPKKYGGFDSPTVAYSVLVVAKVEKGKSKKLKSVKELLGITIMERSSFEKNPIDFLEAKGYKEVKKDLIIKLPKYSLFELENGRKRMLASAGELQKGNELALPSKYVNFLYLASHYEKLKGSPEDNEQKQLFVEQHKHYLDEIIEQISEFSKRVILADANLDKVLSAYNKHRDKPIREQAENIIHLFTLTNLGAPAAFKYFDTTIDRKRYTSTKEVLDATLIHQSITGLYETRIDLSQLGGDAYPYDVPDYASLGSGSPKKKRKVEDPKKKRKVDV

SEQ ID NO: 38 - protein, 1470 aa, synthetic construct
  REGION 1..1470: note = PIN-XTEN-dCas9(delta HNH)-2xNLS
QMELEIRPLFLVPDTNGFIDHLASLARLLESRKYILVVPLIVINELDGLAKGQETDHRAGGYARVVQEKARKSIEFLEQRFESRDSCLRALTSRGNELESIAFRSEDITGQLGNNDDLILSCCLHYCKDKAKDFMPASKEEPIRLLREVVLLTDDRNLRVKALTRNVPVRDIPAFLTWAQVGSGSETPGTSESATPESDKKYSIGLAIGTNSVGWAVITDEYKVPSKKFKVLGNTDRHSIKKNLIGALLFDSGETAEATRLKRTARRRYTRRKNRICYLQEIFSNEMAKVDDSFFHRLEESFLVEEDKKHERHPIFGNIVDEVAYHEKYPTIYHLRKKLVDSTDKADLRLIYLALAHMIKFRGHFLIEGDLNPDNSDVDKLFIQLVQTYNQLFEENPINASGVDAKAILSARLSKSRRLENLIAQLPGEKKNGLFGNLIALSLGLTPNFKSNFDLAEDAKLQLSKDTYDDDLDNLLAQIGDQYADLFLAAKNLSDAILLSDILRVNTEITKAPLSASMIKRYDEHHQDLTLLKALVRQQLPEKYKEIFFDQSKNGYAGYIDGGASQEEFYKFIKPILEKMDGTEELLVKLNREDLLRKQRTFDNGSIPHQIHLGELHAILRRQEDFYPFLKDNREKIEKILTFRIPYYVGPLARGNSRFAWMTRKSEETITPWNFEEVVDKGASAQSFIERMTNFDKNLPNEKVLPKHSLLYEYFTVYNELTKVKYVTEGMRKPAFLSGEQKKAIVDLLFKTNRKVTVKQLKEDYFKKIECFDSVEISGVEDRFNASLGTYHDLLKIIKDKDFLDNEENEDILEDIVLTLTLFEDREMIEERLKTYAHLFDDKVMKQLKRRRYTGWGRLSRKLINGIRDKQSGKTILDFLKSDGFANRNFMQLIHDDSLTFKEDIQKAQVSGQGDSLHEHIANLAGSPAIKKGILQTVKVVDELVKVMGRHKPENIVIEMARENQTTQKGQKNGSGSGLDKAGFIKRQLVETRQITKHVAQILDSRMNTKYDENDKLIREVKVITLKSKLVSDFRKDFQFYKVREINNYHHAHDAYLNAVVGTALIKKYPKLESEFVYGDYKVYDVRKMIAKSEQEIGKATAKYFFYSNIMNFFKTEITLANGEIRKRPLIETNGETGEIVWDKGRDFATVRKVLSMPQVNIVKKTEVQTGGFSKESILPKRNSDKLIARKKDWDPKKYGGFDSPTVAYSVLVVAKVEKGKSKKLKSVKELLGITIMERSSFEKNPIDFLEAKGYKEVKKDLIIKLPKYSLFELENGRKRMLASAGELQKGNELALPSKYVNFLYLASHYEKLKGSPEDNEQKQLFVEQHKHYLDEIIEQISEFSKRVILADANLDKVLSAYNKHRDKPIREQAENIIHLFTLTNLGAPAAFKYFDTTIDRKRYTSTKEVLDATLIHQSITGLYETRIDLSQLGGDAYPYDVPDYASLGSGSPKKKRKVEDPKKKRKVDV

SEQ ID NO: 39 - protein, 1354 aa, synthetic construct
  REGION 1..1354: note = Streptococcus pyogenes dCas9 (D10A, H840A)
MDKKYSIGLAIGTNSVGWAVITDEYKVPSKKFKVLGNTDRHSIKKNLIGALLFDSGETAEATRLKRTARRRYTRRKNRICYLQEIFSNEMAKVDDSFFHRLEESFLVEEDKKHERHPIFGNIVDEVAYHEKYPTIYHLRKKLVDSTDKADLRLIYLALAHMIKFRGHFLIEGDLNPDNSDVDKLFIQLVQTYNQLFEENPINASGVDAKAILSARLSKSRRLENLIAQLPGEKKNGLFGNLIALSLGLTPNFKSNFDLAEDAKLQLSKDTYDDDLDNLLAQIGDQYADLFLAAKNLSDAILLSDILRVNTEITKAPLSASMIKRYDEHHQDLTLLKALVRQQLPEKYKEIFFDQSKNGYAGYIDGGASQEEFYKFIKPILEKMDGTEELLVKLNREDLLRKQRTFDNGSIPHQIHLGELHAILRRQEDFYPFLKDNREKIEKILTFRIPYYVGPLARGNSRFAWMTRKSEETITPWNFEEVVDKGASAQSFIERMTNFDKNLPNEKVLPKHSLLYEYFTVYNELTKVKYVTEGMRKPAFLSGEQKKAIVDLLFKTNRKVTVKQLKEDYFKKIECFDSVEISGVEDRFNASLGTYHDLLKIIKDKDFLDNEENEDILEDIVLTLTLFEDREMIEERLKTYAHLFDDKVMKQLKRRRYTGWGRLSRKLINGIRDKQSGKTILDFLKSDGFANRNFMQLIHDDSLTFKEDIQKAQVSGQGDSLHEHIANLAGSPAIKKGILQTVKVVDELVKVMGRHKPENIVIEMARENQTTQKGQKNSRERMKRIEEGIKELGSQILKEHPVENTQLQNEKLYLYYLQNGRDMYVDQELDINRLSDYDVDAIVPQSFLKDDSIDNKVLTRSDKNRGKSDNVPSEEVVKKMKNYWRQLLNAKLITQRKFDNLTKAERGGLSELDKAGFIKRQLVETRQITKHVAQILDSRMNTKYDENDKLIREVKVITLKSKLVSDFRKDFQFYKVREINNYHHAHDAYLNAVVGTALIKKYPKLESEFVYGDYKVYDVRKMIAKSEQEIGKATAKYFFYSNIMNFFKTEITLANGEIRKRPLIETNGETGEIVWDKGRDFATVRKVLSMPQVNIVKKTEVQTGGFSKESILPKRNSDKLIARKKDWDPKKYGGFDSPTVAYSVLVVAKVEKGKSKKLKSVKELLGITIMERSSFEKNPIDFLEAKGYKEVKKDLIIKLPKYSLFELENGRKRMLASAGELQKGNELALPSKYVNFLYLASHYEKLKGSPEDNEQKQLFVEQHKHYLDEIIEQISEFSKRVILADANLDKVLSAYNKHRDKPIREQAENIIHLFTLTNLGAPAAFKYFDTTIDRKRYTSTKEVLDATLIHQSITG